European Patent Application EP 4 752 156 A1, published June 3, 2026. Title: 抗体及其应用. Applicant: 上海筠璇生物科技有限公司. The sequence listing filed with the application follows.

SEQUENCE LISTING (418 sequences)

SEQ ID NO: 1 - protein, 29 aa, synthetic construct
MEEPGVTPQPYLGLLLEELRRVVAALPEG

SEQ ID NO: 2 - protein, 17 aa, synthetic construct
MELKSPEEEVVAALPEG

SEQ ID NO: 3 - protein, 443 aa, synthetic construct
QIQLVQSGPELKKPGETVKISCKASGYTFTNYAVNWVIQAPGKGLKWMGWINAYTGEPTYADDFKGRFAFSLETSASTAYLQINNLKNEDMGIYFCARGGYDTYALDYWGQGTSVTVSSAKTTPPSVYPLAPGSAAQTNSMVTLGCLVKGYFPEPVTVTWNSGSLSSGVHTFPAVLQSDLYTLSSSVTVPSSTWPSETVTCNVAHPASSTKVDKKIVPRDCGCKPCICTVPEVSSVFIFPPKPKDVLTITLTPKVTCVVVDISKDDPEVQFSWFVDDVEVHTAQTQPREEQFNSTFRSVSELPIMHQDWLNGKEFKCRVNSAAFPAPIEKTISKTKGRPKAPQVYTIPPPKEQMAKDKVSLTCMITDFFPEDITVEWQWNGQPAENYKNTQPIMDTDGSYFVYSKLNVQKSNWEAGNTFTCSVLHEGLHNHHTEKSLSHSPGK

SEQ ID NO: 4 - protein, 219 aa, synthetic construct
DVVMTQTPLTLSVTIGQPASISCKSSQSLLYSNGKTYLSWFLQRPGQSPKRLIYLVSKLDSGVPDRFTGSGSGTDFTLKISRVEAEDLGVYYCVQGTHFPFTFGSGTKLDIKRADAAPTVSIFPPSSEQLTSGGASVVCFLNNFYPKDINVKWKIDGSERQNGVLNSWTDQDSKDSTYSMSSTLTLTKDEYERHNSYTCEATHKTSTSPIVKSFNRNEC

SEQ ID NO: 5 - protein, 119 aa, synthetic construct
QIQLVQSGPELKKPGETVKISCKASGYTFTNYAVNWVIQAPGKGLKWMGWINAYTGEPTYADDFKGRFAFSLETSASTAYLQINNLKNEDMGIYFCARGGYDTYALDYWGQGTSVTVSS

SEQ ID NO: 6 - protein, 112 aa, synthetic construct
DVVMTQTPLTLSVTIGQPASISCKSSQSLLYSNGKTYLSWFLQRPGQSPKRLIYLVSKLDSGVPDRFTGSGSGTDFTLKISRVEAEDLGVYYCVQGTHFPFTFGSGTKLDIK

SEQ ID NO: 7 - protein, 8 aa, synthetic construct
GYTFTNYA

SEQ ID NO: 8 - protein, 8 aa, synthetic construct
INAYTGEP

SEQ ID NO: 9 - protein, 12 aa, synthetic construct
ARGGYDTYALDY

SEQ ID NO: 10 - protein, 11 aa, synthetic construct
QSLLYSNGKTY

SEQ ID NO: 11 - skipped

SEQ ID NO: 12 - protein, 9 aa, synthetic construct
VQGTHFPFT

SEQ ID NO: 13 - protein, 442 aa, synthetic construct
EVQLQQSGPELVKPGASVKISCKTSGYTFTEYTMHWVKQSHGKTLEWIGGIYPNNSGTRYNQKFRGKATLTADKSSSTAYMELRSLTTEDSAVYYCHRYELYWYFDVWGAGTTVTVSSAKTTPPSVYPLAPGSAAQTNSMVTLGCLVKGYFPEPVTVTWNSGSLSSGVHTFPAVLQSDLYTLSSSVTVPSSTWPSETVTCNVAHPASSTKVDKKIVPRDCGCKPCICTVPEVSSVFIFPPKPKDVLTITLTPKVTCVVVDISKDDPEVQFSWFVDDVEVHTAQTQPREEQFNSTFRSVSELPIMHQDWLNGKEFKCRVNSAAFPAPIEKTISKTKGRPKAPQVYTIPPPKEQMAKDKVSLTCMITDFFPEDITVEWQWNGQPAENYKNTQPIMDTDGSYFVYSKLNVQKSNWEAGNTFTCSVLHEGLHNHHTEKSLSHSPGK

SEQ ID NO: 14 - protein, 218 aa, synthetic construct
DIVLTQSPASLAVSLGQRATISCRASKSVSTAGYSYMHWYQQKPGQPPKLLIYLTSNLESGVPARFSGSGSGTDFTLNIHPVEEEDAATYYCQHSREVPYTFGGGTKLEIKRADAAPTVSIFPPSSEQLTSGGASVVCFLNNFYPKDINVKWKIDGSERQNGVLNSWTDQDSKDSTYSMSSTLTLTKDEYERHNSYTCEATHKTSTSPIVKSFNRNEC

SEQ ID NO: 15 - protein, 118 aa, synthetic construct
EVQLQQSGPELVKPGASVKISCKTSGYTFTEYTMHWVKQSHGKTLEWIGGIYPNNSGTRYNQKFRGKATLTADKSSSTAYMELRSLTTEDSAVYYCHRYELYWYFDVWGAGTTVTVSS

SEQ ID NO: 16 - protein, 111 aa, synthetic construct
DIVLTQSPASLAVSLGQRATISCRASKSVSTAGYSYMHWYQQKPGQPPKLLIYLTSNLESGVPARFSGSGSGTDFTLNIHPVEEEDAATYYCQHSREVPYTFGGGTKLEIK

SEQ ID NO: 17 - protein, 8 aa, synthetic construct
GYTFTEYT

SEQ ID NO: 18 - protein, 8 aa, synthetic construct
IYPNNSGT

SEQ ID NO: 19 - protein, 11 aa, synthetic construct
HRYELYWYFDV

SEQ ID NO: 20 - protein, 10 aa, synthetic construct
KSVSTAGYSY

SEQ ID NO: 21 - skipped

SEQ ID NO: 22 - protein, 9 aa, synthetic construct
QHSREVPYT

SEQ ID NO: 23 - protein, 119 aa, synthetic construct
QVQLVQSGSELKKPGASVKISCKASGYTFTNYAVNWVRQAPGQGLEWMGWINAYTGEPTYAQDFTGRFVFSLDTSVSTAYLQINNLKAEDTAIYFCARGGYDTYALDYWGQGTLVTVSS

SEQ ID NO: 24 - protein, 112 aa, synthetic construct
DVVMTQSPLSLPVTPGQPASISCRSSQSLLYSNGKTYLSWFLQRPGQSPRRLIYLVSKRDSGVPDRFSGSGSGTDFTLKISRVEAEDVGVYYCVQGTHFPFTFGQGTKLDIK

SEQ ID NO: 25 - protein, 119 aa, synthetic construct
QVQLVQSGSELKKPGASVKVSCKASGYTFTNYAMNWVRQAPGQGLEWMGWINAYTGEPTYAQGFTGRFVFSLDTSVSTAYLQISSLKAEDTAVYYCARGGYDTYALDYWGQGTTVTVSS

SEQ ID NO: 26 - protein, 112 aa, synthetic construct
DVVMTQSPLSLPVTLGQPASISCRSSQSLLYSNGKTYLNWFQQRPGQSPRRLIYLVSNRDSGVPDRFSGSGSGTDFTLKISRVEAEDVGVYYCVQGTHFPFTFGPGTKVDIK

SEQ ID NO: 27 - protein, 118 aa, synthetic construct
QVQLVQSGAEVKKPGASVKVSCKTSGYTFTEYTMHWVRQAPGQGLEWMGWIYPNNSGTNYAQKFQGRVTLTADTSTSTAYMELRSLTSDDTAVYYCHRYELYWYFDVWGRGTLVTVSS

SEQ ID NO: 28 - protein, 111 aa, synthetic construct
DIVLTQSPASLAVSPGERATISCRASKSVSTAGYSYLHWYQQKPGQPPKLLIYLTSNRASGVPDRFSGSGSGTDFTLTISRVEAEDVAVYYCQHSREVPYTFGQGTKLEIK

SEQ ID NO: 29 - protein, 118 aa, synthetic construct
QVQLVQSGAEVKKPGASVKVSCKASGYTFTEYTMHWVRQAPGQRLEWMGWIYPNNSGTKYSQKFQGRVTITRDTSASTAYMELSSLRSEDTAVYYCHRYELYWYFDVWGRGTLVTVSS

SEQ ID NO: 30 - protein, 111 aa, synthetic construct
DIVLTQSPASLAVSPGQRATITCRASKSVSTAGYSYIHWYQQKPGQPPKLLIYLTSNKDTGVPARFSGSGSGTDFTLTINPVEANDTANYYCQHSREVPYTFGQGTKLEIK

SEQ ID NO: 31 - protein, 119 aa, synthetic construct
EVQLVESGGGLVKPGGSLRLSCAASGFTFSSYSMSWVRQAPGKGLEWVSSISSRSNYIYYADSVKGRFTISRDNAKNSLYLQVNSLRAEDTAVYYCARGSGSYYVFDYWGQGTLVTVSS

SEQ ID NO: 32 - protein, 108 aa, synthetic construct
EIVMTQSPATLSVSPGDRATLSCRASQSISSDLAWYQQKPGQAPRLLIYAASTRATGFPARFSGSGSGTEFTLTISSLQPEDFAVYYCQQYNNWPMYAFGQGTKLEIK

SEQ ID NO: 33 - protein, 8 aa, synthetic construct
GFTFSSYS

SEQ ID NO: 34 - protein, 8 aa, synthetic construct
ISSRSNYI

SEQ ID NO: 35 - protein, 12 aa, synthetic construct
ARGSGSYYVFDY

SEQ ID NO: 36 - protein, 6 aa, synthetic construct
QSISSD

SEQ ID NO: 37 - skipped

SEQ ID NO: 38 - protein, 10 aa, synthetic construct
QQYNNWPMYA

SEQ ID NO: 39 - protein, 113 aa, synthetic construct
QVQLVESGGGLVKPGGSLRLSCAASGFTFSAHYMSWIRQAPGKGLEWVSYISPSSSYTVYADSVKGRFTISRDNAKNSLFLQMNSLRAEDTAVYYCAREGSPGGQGTLVTVSS

SEQ ID NO: 40 - protein, 112 aa, synthetic construct
DVVMTQSPLSLPVTLGQPASISCRPSQSLVDSDGNTYLSWFQQRPGQSPRRLIYKVSDRDSGVPDRFSGSGSVTDFTLKISRVEAEDVGIYYCMQGTHWPFTFGPGTKVDIK

SEQ ID NO: 41 - protein, 8 aa, synthetic construct
GFTFSAHY

SEQ ID NO: 42 - protein, 8 aa, synthetic construct
ISPSSSYT

SEQ ID NO: 43 - protein, 6 aa, synthetic construct
AREGSP

SEQ ID NO: 44 - protein, 11 aa, synthetic construct
QSLVDSDGNTY

SEQ ID NO: 45 - skipped

SEQ ID NO: 46 - protein, 9 aa, synthetic construct
MQGTHWPFT

SEQ ID NO: 47 - protein, 116 aa, synthetic construct
QVQLVQSGAEVKQPGASVKVSCKASGYTFTSYAMHWVRQAPGQRLEWMGWIHAGMGVTKSSQKFQGRITITRDTSASTAYMELSSLRSEDTAVYSCVRQQLGFDYWGQGTLVTVSS

SEQ ID NO: 48 - protein, 112 aa, synthetic construct
DIVMTQSPLSLPVTPGEPASIFCRSSQSLLHSNGNKYLDWYLQKPGQSPQLLIYLGSNRASGVPDRFSGSGSGTDFTLKISRVEAEDVGVYYCMQALQTPYTFGQGTKLEIK

SEQ ID NO: 49 - protein, 8 aa, synthetic construct
GYTFTSYA

SEQ ID NO: 50 - protein, 8 aa, synthetic construct
IHAGMGVT

SEQ ID NO: 51 - protein, 9 aa, synthetic construct
VRQQLGFDY

SEQ ID NO: 52 - protein, 11 aa, synthetic construct
QSLLHSNGNKY

SEQ ID NO: 53 - skipped

SEQ ID NO: 54 - protein, 9 aa, synthetic construct
MQALQTPYT

SEQ ID NO: 55 - protein, 113 aa, synthetic construct
QVQLVESGGGLVKPGGSLRLSCAASGFTFSDHYMSWIRQTPGKGLEWVSYISSSGTYTNYADSVKGRFIISRDNAKNSLFLQMNSLRAEDTAVYYCAREGSPGGQGTLVTVSS

SEQ ID NO: 56 - protein, 112 aa, synthetic construct
DVVMTQSPLSLPVTLGQPASISCRSSQSLVFSDGNTYLNWFQQRPGQSPRRLIYKVSDRDPGVPERFSGSGSGTDFTLKISRVEAEDIGVYYCMQGSHWPFTFGPGTKVDIK

SEQ ID NO: 57 - protein, 8 aa, synthetic construct
GFTFSDHY

SEQ ID NO: 58 - protein, 8 aa, synthetic construct
ISSSGTYT

SEQ ID NO: 59 - protein, 6 aa, synthetic construct
AREGSP

SEQ ID NO: 60 - protein, 11 aa, synthetic construct
QSLVFSDGNTY

SEQ ID NO: 61 - skipped

SEQ ID NO: 62 - protein, 9 aa, synthetic construct
MQGSHWPFT

SEQ ID NO: 63 - protein, 113 aa, synthetic construct
QVQLVESGGGLVKPGGSLRLSCAASGFTFSDHYMSWIRQAPGKGLEWVAYISSSSTYTKYGDSVKGRFTISRDNAKNSLYLQMNSLRAEDTAVYYCAREGSPGGQGTLVTVSS

SEQ ID NO: 64 - protein, 112 aa, synthetic construct
DVVMTQSPLSLPVTLGQPASISCRSSQSLVFSDGNTYLSWFQQRPGQSPRRLIFKVSDRDSGVPDRFSGSGSGTDFTLKISRMEAEDVGVYYCMQGTQWPFTFGPGTKVDIK

SEQ ID NO: 65 - protein, 8 aa, synthetic construct
GFTFSDHY

SEQ ID NO: 66 - protein, 9 aa, synthetic construct
ISSSSTYTK

SEQ ID NO: 67 - protein, 7 aa, synthetic construct
CAREGSP

SEQ ID NO: 68 - protein, 11 aa, synthetic construct
QSLVFSDGNTY

SEQ ID NO: 69 - skipped

SEQ ID NO: 70 - protein, 9 aa, synthetic construct
MQGTQWPFT

SEQ ID NO: 71 - protein, 117 aa, synthetic construct
QVQLVESGGGLVKPGGTLRLSCEASGFTFSDHYMSWIRQAPGKGLEWVSYISSVSGYINYADSVKGRFTISRDNAKKSLYLQMNSLRAEDTAVYYCARGGERFFDYWGQGTLVTVSS

SEQ ID NO: 72 - protein, 113 aa, synthetic construct
DIVMTQSPDSLAVSLGERATINCKSSQSVLYNFNNKIYLAWYQQKPGQPPKLLISWASTRESGVPDRFSGSGSGTDFTLTISSLQAEDVAVYYCQQHYSTPLTFGGGTKVEIK

SEQ ID NO: 73 - protein, 8 aa, synthetic construct
GFTFSDHY

SEQ ID NO: 74 - protein, 8 aa, synthetic construct
ISSVSGYI

SEQ ID NO: 75 - protein, 10 aa, synthetic construct
ARGGERFFDY

SEQ ID NO: 76 - protein, 12 aa, synthetic construct
QSVLYNFNNKIY

SEQ ID NO: 77 - skipped

SEQ ID NO: 78 - protein, 9 aa, synthetic construct
QQHYSTPLT

SEQ ID NO: 79 - protein, 117 aa, synthetic construct; identical to SEQ ID NO: 71

SEQ ID NO: 80 - protein, 113 aa, synthetic construct
DIVMTQSPDSLAVSLGERATINCKSSQNVLYNFNDKNYLAWYQQKPGQPPKLLISWASTRESGVPDRFSGSGSGTDFTLTISSLQAEDVAVYYCQQHYSTPLTFGGGTKVEIK

SEQ ID NO: 81 - protein, 8 aa, synthetic construct
GFTFSDHY

SEQ ID NO: 82 - protein, 8 aa, synthetic construct
ISSVSGYI

SEQ ID NO: 83 - protein, 10 aa, synthetic construct
ARGGERFFDY

SEQ ID NO: 84 - protein, 12 aa, synthetic construct
QNVLYNFNDKNY

SEQ ID NO: 85 - skipped

SEQ ID NO: 86 - protein, 9 aa, synthetic construct
QQHYSTPLT

SEQ ID NO: 87 - protein, 117 aa, synthetic construct
QVQLVESGGGLVKPGGSLRLSCEASGFTFSDHYMSWIRQAPGKGLEWVSYISSSSGYTNYADSVKGRFTISRDNAKNSLYLQMNSLRAEDTAVYYCARGGERFFDYWGQGTLVTVSS

SEQ ID NO: 88 - protein, 113 aa, synthetic construct
DIVMTQSPDSLAVSLGERATINCKSSQSVLYSFNNKNYLAWYQQKPGQPPKLLIYWASTRESGVPDRFSGSGSGTDFTLTISSLQAEDVAVYYCQQHYSTPLTFGGGTKVEIK

SEQ ID NO: 89 - protein, 8 aa, synthetic construct
GFTFSDHY

SEQ ID NO: 90 - protein, 8 aa, synthetic construct
ISSSSGYT

SEQ ID NO: 91 - protein, 10 aa, synthetic construct
ARGGERFFDY

SEQ ID NO: 92 - protein, 12 aa, synthetic construct
QSVLYSFNNKNY

SEQ ID NO: 93 - skipped

SEQ ID NO: 94 - protein, 9 aa, synthetic construct
QQHYSTPLT

SEQ ID NO: 95 - protein, 117 aa, synthetic construct
QVQLVESGGGLVKPGGSLRLSCEASGFTFSDHYMSWIRQAPGKGLEWVSYISSSSGYTNYADSVKGRFTISRDNAKKSLYLQMNSLRAEDTAVYYCARGGERFFDYWGQGTLVTVSS

SEQ ID NO: 96 - protein, 113 aa, synthetic construct
DIVMTQSPDSLAVSLGERATINCKSSQSVLYSFNNKNYLAWYQQKSGQPPKLLISWASTRESGVPDRFSGSGSGTDFTLTISSLQAEDVAVYYCQQHYSTPLTFGGGTKVEIK

SEQ ID NO: 97 - protein, 8 aa, synthetic construct
GFTFSDHY

SEQ ID NO: 98 - protein, 8 aa, synthetic construct
ISSSSGYT

SEQ ID NO: 99 - protein, 10 aa, synthetic construct
ARGGERFFDY

SEQ ID NO: 100 - protein, 12 aa, synthetic construct
QSVLYSFNNKNY

SEQ ID NO: 101 - skipped

SEQ ID NO: 102 - protein, 9 aa, synthetic construct
QQHYSTPLT

SEQ ID NO: 103 - protein, 113 aa, synthetic construct
QVQLVESGGGLVKPGGSLRLSCEASGFTFSAHYMSWIRQAPGKGLEYVSYISSSSSYTNYVDSVKGRFTISRDNAKNSLYLQMNSLRVEDTAVYYCAREGSPGGQGTLVTVSS

SEQ ID NO: 104 - protein, 112 aa, synthetic construct
DVVLTQSPLSLPVTLGQPASISCRSSQSLVDSDGNTYLSWFHQRPGQSPRRLIYKVSDRDSGVPDRFSGSGSGTDFTLKISRVEAEDVGVYYCMEGTHWPFTFGPGTKVDIK

SEQ ID NO: 105 - protein, 8 aa, synthetic construct
GFTFSAHY

SEQ ID NO: 106 - protein, 8 aa, synthetic construct
ISSSSSYT

SEQ ID NO: 107 - protein, 6 aa, synthetic construct
AREGSP

SEQ ID NO: 108 - protein, 11 aa, synthetic construct
QSLVDSDGNTY

SEQ ID NO: 109 - skipped

SEQ ID NO: 110 - protein, 9 aa, synthetic construct
MEGTHWPFT

SEQ ID NO: 111 - protein, 113 aa, synthetic construct
QVQLVESGGGLVKPGGSLRLSCEASGFTFSAHYMSWIRQAPGKGLEYVSYISGSSSYTNYVDSVKGRFTISRDNAKNSLYLQMNSLRVEDTAVYYCAREGSPGGQGTLVTVSS

SEQ ID NO: 112 - protein, 112 aa, synthetic construct; identical to SEQ ID NO: 104

SEQ ID NO: 113 - protein, 8 aa, synthetic construct
GFTFSAHY

SEQ ID NO: 114 - protein, 8 aa, synthetic construct
ISGSSSYT

SEQ ID NO: 115 - protein, 6 aa, synthetic construct
AREGSP

SEQ ID NO: 116 - protein, 11 aa, synthetic construct
QSLVDSDGNTY

SEQ ID NO: 117 - skipped

SEQ ID NO: 118 - protein, 9 aa, synthetic construct
MEGTHWPFT

SEQ ID NO: 119 - protein, 113 aa, synthetic construct
QVQLVESGGGLVKPGGSLRLSCAASGFSFSDSYMSWLRQAPGKGLEWVSYISSSSSYTKYTDSVKGRFTISRDNAKNSLYLQMSSLRAEDTAVYYCAREGSPGGQGTLVTVSS

SEQ ID NO: 120 - protein, 112 aa, synthetic construct
DVVMTQSPLSLPVTLGQPASFSCRSSQSLVFTDGNTFLSWFLQRPGQSPRRLIYRVSNRDPGVPDRFSGSGSGTDFTLKISRVEAEDVGVYYCMQGTQWPFTFGPGTKVDIK

SEQ ID NO: 121 - protein, 8 aa, synthetic construct
GFSFSDSY

SEQ ID NO: 122 - protein, 8 aa, synthetic construct
ISSSSSYT

SEQ ID NO: 123 - protein, 6 aa, synthetic construct
AREGSP

SEQ ID NO: 124 - protein, 11 aa, synthetic construct
QSLVFTDGNTF

SEQ ID NO: 125 - skipped

SEQ ID NO: 126 - protein, 9 aa, synthetic construct
MQGTQWPFT

SEQ ID NO: 127 - protein, 113 aa, synthetic construct
QVQLVESGGGLVKPGGSLRLSCAASGFSFSDSYMSWLRQAPGKGLEWVSYISSSSSYTKYADSVKGRFTISRDNAKNSLYLQMNSLRAEDTAVYYCAREGSPGGQGTLVTVSS

SEQ ID NO: 128 - protein, 112 aa, synthetic construct
DVVLTQSPLSLPVTLGQPASFSCRSSQSLVFTDGNTFLSWFLQRPGQSPRRLIYRVSNRDPGVPDRFSGSGSGTDFTLKISRVEAEDVGVYYCMQGTQWPFTFGPGTKVDIK

SEQ ID NO: 129 - protein, 8 aa, synthetic construct
GFSFSDSY

SEQ ID NO: 130 - protein, 8 aa, synthetic construct
ISSSSSYT

SEQ ID NO: 131 - protein, 6 aa, synthetic construct
AREGSP

SEQ ID NO: 132 - protein, 11 aa, synthetic construct
QSLVFTDGNTF

SEQ ID NO: 133 - skipped

SEQ ID NO: 134 - protein, 9 aa, synthetic construct
MQGTQWPFT

SEQ ID NO: 135 - protein, 113 aa, synthetic construct
QVQLVESGGGLVEPGGSLRLSCAASGFTFSDHYMSWIRQAPGRGLEWVSYISNSGGYTNYADSVKGRFTISRDNAKNSLYLQMNSLRAEDTAVYYCAREGSPGGQGTLVTVSS

SEQ ID NO: 136 - protein, 112 aa, synthetic construct
DVVMTQSPLSLPVTLGQPASMSCRSSQSLVDSDGNTYLSWFQQRPGQSPRRLIYKVSDRDSGVPDRFSGGGSGTDFTLKISRVEAEDVGIYYCMQGTRWPFTFGPGTKVDIK

SEQ ID NO: 137 - protein, 8 aa, synthetic construct
GFTFSDHY

SEQ ID NO: 138 - protein, 8 aa, synthetic construct
ISNSGGYT

SEQ ID NO: 139 - protein, 6 aa, synthetic construct
AREGSP

SEQ ID NO: 140 - protein, 11 aa, synthetic construct
QSLVDSDGNTY

SEQ ID NO: 141 - skipped

SEQ ID NO: 142 - protein, 9 aa, synthetic construct
MQGTRWPFT

SEQ ID NO: 143 - protein, 113 aa, synthetic construct
QVQLVESGGGLVRPGGSLRLSCAASGFTFSDHYMSWIRQAPGKGLEWVSYISGSSSYTKYADSVKGRFTISRDNAKNSLYLQMNSLRAEDTAVYYCAREGSPGGQGTLVTVSS

SEQ ID NO: 144 - protein, 112 aa, synthetic construct
DVVLTQSPLSLPVTLGQPASISCRSSQSLVFSDGNTFLAWFQQRPGQSPRRLIYRISNRDSGVPDRFSGSGSDTDFTLKISRVEAEDVGVYYCMQGTQWPFTFGPGTKVDIK

SEQ ID NO: 145 - protein, 8 aa, synthetic construct
GFTFSDHY

SEQ ID NO: 146 - protein, 8 aa, synthetic construct
ISGSSSYT

SEQ ID NO: 147 - protein, 6 aa, synthetic construct
AREGSP

SEQ ID NO: 148 - protein, 11 aa, synthetic construct
QSLVFSDGNTF

SEQ ID NO: 149 - skipped

SEQ ID NO: 150 - protein, 9 aa, synthetic construct
MQGTQWPFT

SEQ ID NO: 151 - protein, 113 aa, synthetic construct
QVQLVESGGGLVKPGGSLRLSCEASGFTFSAHYMSWIRQAPGKGLEYVSYISSSSSYTNYADSVKGRFTISRDNAKNSLYLQMNSLRAEDTAVYYCAREGSPGGQGTLVTVSS

SEQ ID NO: 152 - protein, 112 aa, synthetic construct; identical to SEQ ID NO: 104

SEQ ID NO: 153 - protein, 8 aa, synthetic construct
GFTFSAHY

SEQ ID NO: 154 - protein, 8 aa, synthetic construct
ISSSSSYT

SEQ ID NO: 155 - protein, 6 aa, synthetic construct
AREGSP

SEQ ID NO: 156 - protein, 11 aa, synthetic construct
QSLVDSDGNTY

SEQ ID NO: 157 - skipped

SEQ ID NO: 158 - protein, 9 aa, synthetic construct
MEGTHWPFT

SEQ ID NO: 159 - protein, 113 aa, synthetic construct; identical to SEQ ID NO: 135

SEQ ID NO: 160 - protein, 112 aa, synthetic construct
DVVMTQSPLSLPVTLGQPASMSCRSSQSLVDSDGNTYLSWFQQRPGQSPRRLIYKVSDRDSGVPDRFSGGGSGTDFTLKIRRVEAEDVGIYYCMQGTRWPFTFGPGTKVDIK

SEQ ID NO: 161 - protein, 8 aa, synthetic construct
GFTFSDHY

SEQ ID NO: 162 - protein, 8 aa, synthetic construct
ISNSGGYT

SEQ ID NO: 163 - protein, 6 aa, synthetic construct
AREGSP

SEQ ID NO: 164 - protein, 11 aa, synthetic construct
QSLVDSDGNTY

SEQ ID NO: 165 - skipped

SEQ ID NO: 166 - protein, 9 aa, synthetic construct
MQGTRWPFT

SEQ ID NO: 167 - protein, 113 aa, synthetic construct
QVQLVESGGGLVKPGGSLRLSCAASGFTFSASYMSWIRQAPGKGLEWVSYISSSSTYTNYADSVKGRFTISRDNAKNSLYLQMDSLRAEDTAMYFCAREGSPGGQGTLVTVSS

SEQ ID NO: 168 - protein, 112 aa, synthetic construct
DVVMTQSPLSLPVTLGQSASISCRSSQSLVYSDGDTFLSWFQQRPGQSPRRLIYMVSNRDPGVPDRFSGSGSGTDFTLKISRVEAEDVGIYYCMQGTNWPFTFGPGTRVDIK

SEQ ID NO: 169 - protein, 8 aa, synthetic construct
GFTFSASY

SEQ ID NO: 170 - protein, 8 aa, synthetic construct
ISSSSTYT

SEQ ID NO: 171 - protein, 6 aa, synthetic construct
AREGSP

SEQ ID NO: 172 - protein, 11 aa, synthetic construct
QSLVYSDGDTF

SEQ ID NO: 173 - skipped

SEQ ID NO: 174 - protein, 9 aa, synthetic construct
MQGTNWPFT

SEQ ID NO: 175 - protein, 113 aa, synthetic construct
QVQLVESGGGLVKPGGSLRLSCAASGFSFSDSYMSWIRQAPGKGLEWVSYISSSSSYTNYADSVKGRFTISRDNAKNSLYLQMNSLRVEDTAVYYCAREGSPGGQGTLVTVSS

SEQ ID NO: 176 - protein, 112 aa, synthetic construct
DVVLTQSPLSLPVTLGQPASISCRSSQSLVDSDGNTYLSWFQQRPGQSPRRLIYRVSNRDSGVPDRFSGSGSGTDFTLKISRVEAEDVGVYYCMQGTHWPFTFGPGTKVDIK

SEQ ID NO: 177 - protein, 8 aa, synthetic construct
GFSFSDSY

SEQ ID NO: 178 - protein, 8 aa, synthetic construct
ISSSSSYT

SEQ ID NO: 179 - protein, 6 aa, synthetic construct
AREGSP

SEQ ID NO: 180 - protein, 11 aa, synthetic construct
QSLVDSDGNTY

SEQ ID NO: 181 - skipped

SEQ ID NO: 182 - protein, 9 aa, synthetic construct
MQGTHWPFT

SEQ ID NO: 183 - protein, 113 aa, synthetic construct
QVQLVESGGGLVKPGGSLRLSCAASGFSFSDSYMSWIRQAPGKGLEWVSYISSSSSYTNYVDSVKGRFTISRDNAKNSLYLQMNSLRVEDTAVYYCAREGSPGGQGTLVTVSS

SEQ ID NO: 184 - protein, 112 aa, synthetic construct
DVVMTQSPLSLPVTLGQPASISCRSSQSLVDSDGNTYLSWFQQRPGQSPRRLIYRVSNRDSGVPDRFSGSGSGTDFTLKISRVEAEDVGVYYCMQGTHWPFTFGPGTKVDIR

SEQ ID NO: 185 - protein, 8 aa, synthetic construct
GFSFSDSY

SEQ ID NO: 186 - protein, 8 aa, synthetic construct
ISSSSSYT

SEQ ID NO: 187 - protein, 6 aa, synthetic construct
AREGSP

SEQ ID NO: 188 - protein, 11 aa, synthetic construct
QSLVDSDGNTY

SEQ ID NO: 189 - skipped

SEQ ID NO: 190 - protein, 9 aa, synthetic construct
MQGTHWPFT

SEQ ID NO: 191 - protein, 113 aa, synthetic construct; identical to SEQ ID NO: 39

SEQ ID NO: 192 - protein, 112 aa, synthetic construct
DVVMTQSPLSLPVTLGQPASISCRSTQSLVDSDGNTYLSWFQQRPGQSPRRLIYKVSDRDSGVPDRFSGSGSGTDFTLKISRVEAEDIGIYYCMQGTHWPFTFGPGTKVDIK

SEQ ID NO: 193 - protein, 8 aa, synthetic construct
GFTFSAHY

SEQ ID NO: 194 - protein, 8 aa, synthetic construct
ISPSSSYT

SEQ ID NO: 195 - protein, 6 aa, synthetic construct
AREGSP

SEQ ID NO: 196 - protein, 11 aa, synthetic construct
QSLVDSDGNTY

SEQ ID NO: 197 - skipped

SEQ ID NO: 198 - protein, 9 aa, synthetic construct
MQGTHWPFT

SEQ ID NO: 199 - protein, 113 aa, synthetic construct; identical to SEQ ID NO: 39

SEQ ID NO: 200 - protein, 112 aa, synthetic construct
DVVMTQSPLSLPVTLGQPASISCRSSQNLVDSDGNTYLSWFQQRPGQSPRRLIYKVSDRDSGVPDRFSGSGSGTDFTLKINRVEAEDIGIYYCMQGSHWPFTFGPGTKVDIK

SEQ ID NO: 201 - protein, 8 aa, synthetic construct
GFTFSAHY

SEQ ID NO: 202 - protein, 8 aa, synthetic construct
ISPSSSYT

SEQ ID NO: 203 - protein, 6 aa, synthetic construct
AREGSP

SEQ ID NO: 204 - protein, 11 aa, synthetic construct
QNLVDSDGNTY

SEQ ID NO: 205 - skipped

SEQ ID NO: 206 - protein, 9 aa, synthetic construct
MQGSHWPFT

SEQ ID NO: 207 - protein, 114 aa, synthetic construct
EVQLVESGGGLVQPGGSLRLSCAASGFTFSSYAMSWVRQAPGKGLEWVSGISGSVDITHHADSVKGRFTISRDNSKNTLYLQMNSLRAEDTAVYYCVRGGFDYWGQGSLVTVSS

SEQ ID NO: 208 - protein, 107 aa, synthetic construct
DIQMTQSPSSVSASVGDRVTISCRASQDISTWLAWYQQKPGKAPRLLIYAASTLLIGVPSRFSGSGSGTDFTLTISSLQPEDFATYYCQQTNSFPITFGQGTRLEIK

SEQ ID NO: 209 - protein, 8 aa, synthetic construct
GFTFSSYA

SEQ ID NO: 210 - protein, 8 aa, synthetic construct
ISGSVDIT

SEQ ID NO: 211 - protein, 7 aa, synthetic construct
VRGGFDY

SEQ ID NO: 212 - protein, 6 aa, synthetic construct
QDISTW

SEQ ID NO: 213 - skipped

SEQ ID NO: 214 - protein, 9 aa, synthetic construct
QQTNSFPIT

SEQ ID NO: 215 - protein, 114 aa, synthetic construct
EVQLVESGGGLVQPGGSLRLSCAASGFTFSSYAMTWVRQAPGKGLEWVSGISGSIGITHHADSVKGRFTISRDNSKNTLYLQMNSLRAEDTAVYYCVRGGFDYWGQGSLVTVSS

SEQ ID NO: 216 - protein, 107 aa, synthetic construct
DIQMTQSPSSVSASVGDRVTITCRASQDINTWLAWYQQKPGKAPKLLIYTSSTLLGGVPSRFSGSGSGTDFTLTISSLQPEDFGTYYCQQTNTFPITFGQGTRLEIK

SEQ ID NO: 217 - protein, 8 aa, synthetic construct
GFTFSSYA

SEQ ID NO: 218 - protein, 8 aa, synthetic construct
ISGSIGIT

SEQ ID NO: 219 - protein, 7 aa, synthetic construct
VRGGFDY

SEQ ID NO: 220 - protein, 6 aa, synthetic construct
QDINTW

SEQ ID NO: 221 - skipped

SEQ ID NO: 222 - protein, 9 aa, synthetic construct
QQTNTFPIT

SEQ ID NO: 223 - protein, 119 aa, synthetic construct
EVQLVESGGGLVKRGGSLRLSCAASGFTFSSYSMHWVRQAPGKGLEWVSSISSRSTYIYYADSVKGRFTISRDNAKNSLYLQMNSLSAEDTAVYYCARGSGSYYVFDYWGQGTLVTVSS

SEQ ID NO: 224 - protein, 108 aa, synthetic construct
ELVMTQSPATLSVSPGERATLSCRASQSVSSNLAWYQQKPGQAPRLLIYGASSRATNIPARFSGSGSGTEFTLTISSLQSEDFAVYYCQQYDNWPMYSFGQGTKLEIK

SEQ ID NO: 225 - protein, 8 aa, synthetic construct
GFTFSSYS

SEQ ID NO: 226 - protein, 8 aa, synthetic construct
ISSRSTYI

SEQ ID NO: 227 - protein, 12 aa, synthetic construct
ARGSGSYYVFDY

SEQ ID NO: 228 - protein, 6 aa, synthetic construct
QSVSSN

SEQ ID NO: 229 - skipped

SEQ ID NO: 230 - protein, 10 aa, synthetic construct
QQYDNWPMYS

SEQ ID NO: 231 - protein, 114 aa, synthetic construct
EVQLVESGGGLVQPGGSLRLSCAASGFTFSSYAMTWVRQAPGKGLEWVSGISGSVGITHHADSVKGRFTISRDNSKNTLYLQMNSLRVEDTAVYYCVRGGFDYWGQGSLVTVSS

SEQ ID NO: 232 - protein, 107 aa, synthetic construct
DIQMTQSPSSVSASVGDRVTITCRASQDINTWLAWYQQKPGKAPKLLIYTTSTLLSGVPSRFSGSGSGTDFTLTISSLQPEDFATYYCQQTNTFPITFGQGTRLEIK

SEQ ID NO: 233 - protein, 8 aa, synthetic construct
GFTFSSYA

SEQ ID NO: 234 - protein, 8 aa, synthetic construct
ISGSVGIT

SEQ ID NO: 235 - protein, 7 aa, synthetic construct
VRGGFDY

SEQ ID NO: 236 - protein, 6 aa, synthetic construct
QDINTW

SEQ ID NO: 237 - skipped

SEQ ID NO: 238 - protein, 9 aa, synthetic construct
QQTNTFPIT

SEQ ID NO: 239 - protein, 119 aa, synthetic construct
EVQLVESGGGLVKPGGSLRLSCAASGFTFSSYSMSWVRQAPGKGLEWVSSISSRSNYIYYADSVKGRITISRDNAKNSLYLQMNSLRAEDTAVYYCARGSGSYYVFDYWGQGTLVTVSS

SEQ ID NO: 240 - protein, 108 aa, synthetic construct
ELVMTQSPATLSMSPGDRATLSCRASQSIRSDLAWYQQKPGQAPRLLIYDASTRATGIPARFSGSGSGTEFTLSISSLQSEDFAVYYCQQYNNWPMYTFGQGTKLEIK

SEQ ID NO: 241 - protein, 8 aa, synthetic construct
GFTFSSYS

SEQ ID NO: 242 - protein, 8 aa, synthetic construct
ISSRSNYI

SEQ ID NO: 243 - protein, 12 aa, synthetic construct
ARGSGSYYVFDY

SEQ ID NO: 244 - protein, 6 aa, synthetic construct
QSIRSD

SEQ ID NO: 245 - skipped

SEQ ID NO: 246 - protein, 10 aa, synthetic construct
QQYNNWPMYT

SEQ ID NO: 247 - protein, 119 aa, synthetic construct
QVQLVESGGGVVQPGRSLRLSCAASGFTFSRYGIHWVRQAPGKGLEWVAVITYDGRKKFYADSVQGRFTISRDNSRNTLSLQMNSLRAEDTAVYYCAKDLLIGYGMDVWGQGTTVTVSS

SEQ ID NO: 248 - protein, 113 aa, synthetic construct
DIVMTQSPDSLAVSLGERATINCKSSQSVLFSSNNKNFLAWYQQKPGQPPKLLIYWASTRESGVPDRFSGSGSGTDFTLTISSLQPEDVALYFCQQCYSTPYTFGQGTKLEIK

SEQ ID NO: 249 - protein, 8 aa, synthetic construct
GFTFSRYG

SEQ ID NO: 250 - protein, 8 aa, synthetic construct
ITYDGRKK

SEQ ID NO: 251 - protein, 12 aa, synthetic construct
AKDLLIGYGMDV

SEQ ID NO: 252 - protein, 12 aa, synthetic construct
QSVLFSSNNKNF

SEQ ID NO: 253 - skipped

SEQ ID NO: 254 - protein, 9 aa, synthetic construct
QQCYSTPYT

SEQ ID NO: 255 - protein, 119 aa, synthetic construct
QVQLVESGGGVVQPGRSLTLSCAASGFTFSRYGMHWVRQAPGKGLEWVTVITYDGRKKYYADSVKGRFTISRDNSQNTLSLQMNSLRAEDTAVYYCAKDLLIGYGMDVWGQGTTVTVSS

SEQ ID NO: 256 - protein, 113 aa, synthetic construct
DIVMTQSPDSLAVSLGERATIKCKSSQSVFFSSSNKNFLTWYQQKPGQPPKLLIYWASTRESGVPDRFSGSGSGTDFTLTINNLQAEDVTVYYCQQCFSTPYSFGQGTKLEIK

SEQ ID NO: 257 - protein, 8 aa, synthetic construct
GFTFSRYG

SEQ ID NO: 258 - protein, 8 aa, synthetic construct
ITYDGRKK

SEQ ID NO: 259 - protein, 12 aa, synthetic construct
AKDLLIGYGMDV

SEQ ID NO: 260 - protein, 12 aa, synthetic construct
QSVFFSSSNKNF

SEQ ID NO: 261 - skipped

SEQ ID NO: 262 - protein, 9 aa, synthetic construct
QQCFSTPYS

SEQ ID NO: 263 - protein, 119 aa, synthetic construct
QVQLVESGGGVVQPGRSLRLSCAASGFTFSRYGIHWVRQAPGKGLEWVAVITYDGRKKFYADSVKGRFTISRDNSRNTLSLQMNSLRAEDTAVYYCAKDLLIGYGMDVWGQGTTVTVSS

SEQ ID NO: 264 - protein, 113 aa, synthetic construct; identical to SEQ ID NO: 248

SEQ ID NO: 265 - protein, 8 aa, synthetic construct
GFTFSRYG

SEQ ID NO: 266 - protein, 8 aa, synthetic construct
ITYDGRKK

SEQ ID NO: 267 - protein, 12 aa, synthetic construct
AKDLLIGYGMDV

SEQ ID NO: 268 - protein, 12 aa, synthetic construct
QSVLFSSNNKNF

SEQ ID NO: 269 - skipped

SEQ ID NO: 270 - protein, 9 aa, synthetic construct
QQCYSTPYT

SEQ ID NO: 271 - protein, 119 aa, synthetic construct
QVQLVESGGGVVQPGRSLRLSCAASGFTFSSYGMHWVRQAPGKGLEWVAVISYDGSNKYYADSVKGRFTISKDNSKNTLYLQMNSLRAEDTAVYYCAKDLLAGYGMDVWGQGTTVTVSS

SEQ ID NO: 272 - protein, 113 aa, synthetic construct
DIVMTQSPDSLAVSLGERATINCKSSQSVLYSSNNKNFLAWYQQKPGQPPKLLIYWASTRESGVPDRFSGSGSGTDFTLTISSLQAEDVAVYYCQQYYSTPYTFGQGTKLEIK

SEQ ID NO: 273 - protein, 8 aa, synthetic construct
GFTFSSYG

SEQ ID NO: 274 - protein, 8 aa, synthetic construct
ISYDGSNK

SEQ ID NO: 275 - protein, 12 aa, synthetic construct
AKDLLAGYGMDV

SEQ ID NO: 276 - protein, 12 aa, synthetic construct
QSVLYSSNNKNF

SEQ ID NO: 277 - skipped

SEQ ID NO: 278 - protein, 9 aa, synthetic construct
QQYYSTPYT

SEQ ID NO: 279 - protein, 119 aa, synthetic construct
QVQLVESGGGVVQPGRSLRLSCAASGFTFSSYGMHWVRQAPGKGLEWVTVITYDGSRKFYADSVKGRFTISRDSSKNTLYLQMNSLRVEDTAVYYCAKDHLRGYGMDVWGQGTTVTVSS

SEQ ID NO: 280 - protein, 113 aa, synthetic construct
DIVMTQSPDSLAVSLGERATINCKSSQSVLFSSNNKNFLAWYQQKPGQPPVLLIKWASTRYSGVPDRFSGSGSGTDFTLTISSLQAEDVAVYYCQQYYSTPYTFGQGTKLEIK

SEQ ID NO: 281 - protein, 8 aa, synthetic construct
GFTFSSYG

SEQ ID NO: 282 - protein, 8 aa, synthetic construct
ITYDGSRK

SEQ ID NO: 283 - protein, 12 aa, synthetic construct
AKDHLRGYGMDV

SEQ ID NO: 284 - protein, 12 aa, synthetic construct
QSVLFSSNNKNF

SEQ ID NO: 285 - skipped

SEQ ID NO: 286 - protein, 9 aa, synthetic construct
QQYYSTPYT

SEQ ID NO: 287 - protein, 119 aa, synthetic construct
QVQLVESGGGVVQPGRSLRLSCAASGFTFSRYGIHWVRQAPGKGLEWVAVITYDGRKKYYADSVKGRFTISRDNSQNTLSLQMNSLTTEDTGVYYCAKDLLIGYGMDVWGQGTTVTVSS

SEQ ID NO: 288 - protein, 113 aa, synthetic construct
DIVMTQSPDSLAVSLGERATINCKSSQSVLFSSNKKNFLTWYQQKPGQPPKLLIYWASTRESGVPDRFSGSGSGTDFTLTISSLQAEDVAVYYCQQCYSTPYSFGRGTKLEIK

SEQ ID NO: 289 - protein, 8 aa, synthetic construct
GFTFSRYG

SEQ ID NO: 290 - protein, 8 aa, synthetic construct
ITYDGRKK

SEQ ID NO: 291 - protein, 12 aa, synthetic construct
AKDLLIGYGMDV

SEQ ID NO: 292 - protein, 12 aa, synthetic construct
QSVLFSSNKKNF

SEQ ID NO: 293 - skipped

SEQ ID NO: 294 - protein, 9 aa, synthetic construct
QQCYSTPYS

SEQ ID NO: 295 - protein, 119 aa, synthetic construct
QVQLVESGGGVVQPGRSLRLSCAASGFTFSRYGIHWVRQAPGKGLEWVAVITYDGRKKFYADSVKGRFTISRDNSRNTLSLQMNSLRAEDTAVYYCAKDLLIGYGLDVWGQGTTVTVSS

SEQ ID NO: 296 - protein, 113 aa, synthetic construct
DIVMTQSPDSLAVSLGERATINCKSSQSVLFSSNNKNFLAWYQQKPGQPPKLLIYWASTRESGVPDRFSGSGSGTDFTLTISSLQPEDVALYFCQQCYSTPYSFGQGTKLEIK

SEQ ID NO: 297 - protein, 8 aa, synthetic construct
GFTFSRYG

SEQ ID NO: 298 - protein, 8 aa, synthetic construct
ITYDGRKK

SEQ ID NO: 299 - protein, 12 aa, synthetic construct
AKDLLIGYGLDV

SEQ ID NO: 300 - protein, 12 aa, synthetic construct
QSVLFSSNNKNF

SEQ ID NO: 301 - skipped

SEQ ID NO: 302 - protein, 9 aa, synthetic construct
QQCYSTPYS

SEQ ID NO: 303 - protein, 119 aa, synthetic construct
QVQLVESGGGVVQPGRSLRLSCAASGFTFSSYGMHWVRQAPGKGLEWVTVITYDGSRKFYADSVKGRFTISRDSSKNTLFLQMNSLRVEDTAVYYCAKDHLRGYGMDVWGQGTTVTVSS

SEQ ID NO: 304 - protein, 113 aa, synthetic construct; identical to SEQ ID NO: 280

SEQ ID NO: 305 - protein, 8 aa, synthetic construct
GFTFSSYG

SEQ ID NO: 306 - protein, 8 aa, synthetic construct
ITYDGSRK

SEQ ID NO: 307 - protein, 12 aa, synthetic construct
AKDHLRGYGMDV

SEQ ID NO: 308 - protein, 12 aa, synthetic construct
QSVLFSSNNKNF

SEQ ID NO: 309 - skipped

SEQ ID NO: 310 - protein, 9 aa, synthetic construct
QQYYSTPYT

SEQ ID NO: 311 - protein, 119 aa, synthetic construct
QVQLVESGGGVVQPGRSLRLSCAASGFTFSSYGMHWVRQAPGKGLEWVAVITYDGSKKYYADSVKGRFTISRDNSKNTLYLQMNSLRAEDTAVYYCAKDRAVGYGMDAWGQGTTVTVSS

SEQ ID NO: 312 - protein, 113 aa, synthetic construct
DIVMTQSPDSLAVSLGERATINCKSSQSVLFSSNNKNFLAWYQQKSGQPPKQLIFWASIRESGVPDRFSGSGSGTDFTLTISSLQAEDVAVYSCQQYYSTPYTFGQGTKLEIK

SEQ ID NO: 313 - protein, 8 aa, synthetic construct
GFTFSSYG

SEQ ID NO: 314 - protein, 8 aa, synthetic construct
ITYDGSKK

SEQ ID NO: 315 - protein, 12 aa, synthetic construct
AKDRAVGYGMDA

SEQ ID NO: 316 - protein, 12 aa, synthetic construct
QSVLFSSNNKNF

SEQ ID NO: 317 - skipped

SEQ ID NO: 318 - protein, 9 aa, synthetic construct
QQYYSTPYT

SEQ ID NO: 319 - protein, 119 aa, synthetic construct
QVQLVESGGGVVQPGRSLRLSCAASGFTFSSYGMHWVRQAPGKGLEWVAVITYDGSKKYYADSVKGRFTISKDNSKNTLYLQMNSLRAEDTAVFYCAKDRALGYGMDVWGQGTTVTVSS

SEQ ID NO: 320 - protein, 113 aa, synthetic construct
DIVMTQSPDSLAVSLGERATINCKSSQTVLFSSNNKNFLTWYQQKSGQPPKQIIYWASTRESGVPDRFSGSGSGTDFTLTINSLQAEDVAVYYCQQYFSTPYTFGQGTKLEIK

SEQ ID NO: 321 - protein, 8 aa, synthetic construct
GFTFSSYG

SEQ ID NO: 322 - protein, 8 aa, synthetic construct
ITYDGSKK

SEQ ID NO: 323 - protein, 12 aa, synthetic construct
AKDRALGYGMDV

SEQ ID NO: 324 - protein, 12 aa, synthetic construct
QTVLFSSNNKNF

SEQ ID NO: 325 - skipped

SEQ ID NO: 326 - protein, 9 aa, synthetic construct
QQYFSTPYT

SEQ ID NO: 327 - protein, 119 aa, synthetic construct
QVQLVESGGGVVQPGRSLRLSCAASGFTFNSYGMHWVRQAPGKGLEWVAVISKDGSKKYYADSVKGRFTISRDKSKNTLYLQMNSLRAEDTAVYYCAKDRALGYGMDVWGQGTTVTVSS

SEQ ID NO: 328 - protein, 113 aa, synthetic construct
DIVMTQSPDSLAVSLGERATINCKSSQSVLYSVNNKNFLTWYQQKPGQPPKQLIYWASTRESGVPDRFSGSGSGTDFTLTISSLQAEDVAVYYCQHYYSTPYTFGQGTKLEIK

SEQ ID NO: 329 - protein, 8 aa, synthetic construct
GFTFNSYG

SEQ ID NO: 330 - protein, 8 aa, synthetic construct
ISKDGSKK

SEQ ID NO: 331 - protein, 12 aa, synthetic construct
AKDRALGYGMDV

SEQ ID NO: 332 - protein, 12 aa, synthetic construct
QSVLYSVNNKNF

SEQ ID NO: 333 - skipped

SEQ ID NO: 334 - protein, 9 aa, synthetic construct
QHYYSTPYT

SEQ ID NO: 335 - protein, 119 aa, synthetic construct; identical to SEQ ID NO: 319

SEQ ID NO: 336 - protein, 113 aa, synthetic construct
DIVMTQSPDSLAVSLGERATINCKSSQTVLFSSNNKNFLTWYQQKSGQPPKQIIYWASTRESGVPDRFSGSGSGTDFTLTISSLQAEDVAVYYCQQYFSTPYTFGQGTKLEIK

SEQ ID NO: 337 - protein, 8 aa, synthetic construct
GFTFSSYG

SEQ ID NO: 338 - protein, 8 aa, synthetic construct
ITYDGSKK

SEQ ID NO: 339 - protein, 12 aa, synthetic construct
AKDRALGYGMDV

SEQ ID NO: 340 - protein, 12 aa, synthetic construct
QTVLFSSNNKNF

SEQ ID NO: 341 - skipped

SEQ ID NO: 342 - protein, 9 aa, synthetic construct
QQYFSTPYT

SEQ ID NO: 343 - protein, 119 aa, synthetic construct; identical to SEQ ID NO: 327

SEQ ID NO: 344 - protein, 113 aa, synthetic construct
DIVMTQSPDSLAVSLGERATINCKSSQSVLYSVNNKNFLTWYQQKPGQPPKQLIYWASTRESGVPDRFSGSGSGTDFSLTISGLQAEDVAVYYCQHYYSAPYTFGQGTKLEIK

SEQ ID NO: 345 - protein, 8 aa, synthetic construct
GFTFNSYG

SEQ ID NO: 346 - protein, 8 aa, synthetic construct
ISKDGSKK

SEQ ID NO: 347 - protein, 12 aa, synthetic construct
AKDRALGYGMDV

SEQ ID NO: 348 - protein, 11 aa, synthetic construct
QSVLYSVNNKN

SEQ ID NO: 349 - skipped

SEQ ID NO: 350 - protein, 9 aa, synthetic construct
QHYYSAPYT

SEQ ID NO: 351 - protein, 119 aa, synthetic construct
QVQLVESGGGVVQPGRSLRLSCVASGFTFSSYGMHWVRQAPGKGLEWVAVITYDGSKKYYADSVKGRFTISRDSSKNTLYLQMNSLRAEDTAVYYCAKDRAVGYGMDVWGQGTTVTVSS

SEQ ID NO: 352 - protein, 113 aa, synthetic construct
DIVMTQSPDSLAVSLGERATINCKSSQSVLYRSNNKNFLTWYQQKSGQSPKQLIYWASTRESGVPDRFSGSGSGTDFTLTISSLQAEDVAVYYCQQYYSTPYTFGQGTKLEIK

SEQ ID NO: 353 - protein, 8 aa, synthetic construct
GFTFSSYG

SEQ ID NO: 354 - protein, 8 aa, synthetic construct
ITYDGSKK

SEQ ID NO: 355 - protein, 12 aa, synthetic construct
AKDRAVGYGMDV

SEQ ID NO: 356 - protein, 12 aa, synthetic construct
QSVLYRSNNKNF

SEQ ID NO: 357 - skipped

SEQ ID NO: 358 - protein, 9 aa, synthetic construct
QQYYSTPYT

SEQ ID NO: 359 - protein, 119 aa, synthetic construct
QVQLVESGGGVVQPGRSLRLSCAASGFTFSRYGIHWVRQAPGKGLEWVAVISYHGSNKYYADSVKGRFTISRDNSKNTLYLQMNSLRAEDTAVYYCAKDRALGYGMDVWGQGTTVTVSS

SEQ ID NO: 360 - protein, 113 aa, synthetic construct
DIVVTQSPDSLAVSLGERATINCKSSQSVLFNSNNKNFLTWYQQKPGQPPKQLIYWASTRESGVPDRFSGSGSGTDFTLTISSLQAEDVAVYYCQQYYSTPYAFGQGTKLEIK

SEQ ID NO: 361 - protein, 8 aa, synthetic construct
GFTFSRYG

SEQ ID NO: 362 - protein, 8 aa, synthetic construct
ISYHGSNK

SEQ ID NO: 363 - protein, 12 aa, synthetic construct
AKDRALGYGMDV

SEQ ID NO: 364 - protein, 12 aa, synthetic construct
QSVLFNSNNKNF

SEQ ID NO: 365 - skipped

SEQ ID NO: 366 - protein, 9 aa, synthetic construct
QQYYSTPYA

SEQ ID NO: 367 - protein, 119 aa, synthetic construct
QVQLVESGGGAVQPGRSLRLSCAASGFTFSRYGMHWVRQAPGKGLEWVAVITYDGSKKYYADSVKGRFTISRDNSKNTLSLQMNSLRAEDTAVYYCAKDRALGYGMDVWGQGTTVTVSS

SEQ ID NO: 368 - protein, 113 aa, synthetic construct
DIVMTQSPDSLAVSLGERATINCKSSQSVLYTANNKNFLTWYQQKSGQPPKQLIYWASTRESGVPDRFSGSGSGTDFTLTISSLQAEDVAVYYCQQYYSTPYTFGQGTKLEIK

SEQ ID NO: 369 - protein, 8 aa, synthetic construct
GFTFSRYG

SEQ ID NO: 370 - protein, 8 aa, synthetic construct
ITYDGSKK

SEQ ID NO: 371 - protein, 12 aa, synthetic construct
AKDRALGYGMDV

SEQ ID NO: 372 - protein, 12 aa, synthetic construct
QSVLYTANNKNF

SEQ ID NO: 373 - skipped

SEQ ID NO: 374 - protein, 9 aa, synthetic construct
QQYYSTPYT

SEQ ID NO: 375 - protein, 119 aa, synthetic construct; identical to SEQ ID NO: 351

SEQ ID NO: 376 - protein, 113 aa, synthetic construct; identical to SEQ ID NO: 352

SEQ ID NO: 377 - protein, 8 aa, synthetic construct
GFTFSSYG

SEQ ID NO: 378 - protein, 8 aa, synthetic construct
ITYDGSKK

SEQ ID NO: 379 - protein, 12 aa, synthetic construct
AKDRAVGYGMDV

SEQ ID NO: 380 - protein, 11 aa, synthetic construct
QSVLYRSNNKN

SEQ ID NO: 381 - skipped

SEQ ID NO: 382 - protein, 9 aa, synthetic construct
QQYYSTPYT

SEQ ID NO: 383 - protein, 119 aa, synthetic construct
QVQLVESGGGVVQPGRSLRLSCAASGFTFSSYGMHWVRQAPGKGLEWVAVISYDGSKKYYADSVKGRFTISRDISKNTLYLQMNSLRAEDTAVYYCAKDRALGYGMDVWGQGTTVTVSS

SEQ ID NO: 384 - protein, 113 aa, synthetic construct
DIVMTQSPDSLAVSLGERATINCKSSQSVLYSANNKNFLTWYQQKPGQPPKQLIYWASTRESGVPDRFSGSGSGTDFTLIISSLQAEDVAVYYCQQYYSTPYTFGQGTKLEIK

SEQ ID NO: 385 - protein, 8 aa, synthetic construct
GFTFSSYG

SEQ ID NO: 386 - protein, 8 aa, synthetic construct
ISYDGSKK

SEQ ID NO: 387 - protein, 12 aa, synthetic construct
AKDRALGYGMDV

SEQ ID NO: 388 - protein, 11 aa, synthetic construct
QSVLYSANNKN

SEQ ID NO: 389 - skipped

SEQ ID NO: 390 - protein, 9 aa, synthetic construct
QQYYSTPYT

SEQ ID NO: 391 - protein, 119 aa, synthetic construct; identical to SEQ ID NO: 359

SEQ ID NO: 392 - protein, 113 aa, synthetic construct
DIVVTQSPDSLAVSLGERATINCKSSQSVLFNSNNKNFLTWYQQKPGQPPKQLIYWASTRESGVPDRFSGSGSGTDFTLTISSLQAEDVAIYYCQQYYSTPYAFGQGTKLEIK

SEQ ID NO: 393 - protein, 8 aa, synthetic construct
GFTFSRYG

SEQ ID NO: 394 - protein, 8 aa, synthetic construct
ISYHGSNK

SEQ ID NO: 395 - protein, 12 aa, synthetic construct
AKDRALGYGMDV

SEQ ID NO: 396 - protein, 12 aa, synthetic construct
QSVLFNSNNKNF

SEQ ID NO: 397 - skipped

SEQ ID NO: 398 - protein, 9 aa, synthetic construct
QQYYSTPYA

SEQ ID NO: 399 - protein, 119 aa, synthetic construct; identical to SEQ ID NO: 383

SEQ ID NO: 400 - protein, 113 aa, synthetic construct; identical to SEQ ID NO: 384

SEQ ID NO: 401 - protein, 8 aa, synthetic construct
GFTFSSYG

SEQ ID NO: 402 - protein, 8 aa, synthetic construct
ISYDGSKK

SEQ ID NO: 403 - protein, 12 aa, synthetic construct
AKDRALGYGMDV

SEQ ID NO: 404 - protein, 11 aa, synthetic construct
QSVLYSANNKN

SEQ ID NO: 405 - skipped

SEQ ID NO: 406 - protein, 9 aa, synthetic construct
QQYYSTPYT

SEQ ID NO: 407 - protein, 119 aa, synthetic construct; identical to SEQ ID NO: 327

SEQ ID NO: 408 - protein, 113 aa, synthetic construct; identical to SEQ ID NO: 328

SEQ ID NO: 409 - protein, 8 aa, synthetic construct
GFTFNSYG

SEQ ID NO: 410 - protein, 8 aa, synthetic construct
ISKDGSKK

SEQ ID NO: 411 - protein, 12 aa, synthetic construct
AKDRALGYGMDV

SEQ ID NO: 412 - protein, 11 aa, synthetic construct
QSVLYSVNNKN

SEQ ID NO: 413 - skipped

SEQ ID NO: 414 - protein, 9 aa, synthetic construct
QHYYSTPYT

SEQ ID NO: 415 - protein, 804 aa, synthetic construct
MEEPGVTPQPYLGLLLEELRRVVAALPEGMRPDSNLYGFPWELVICAAVVGFFAVLFFLWRSFRSVRSRLYVGREKKLALMLSGLIEEKSKLLEKFSLVQKEYEGYEVESSLKDASFEKEATEAQSLEATCEKLNRSNSELEDEILCLEKELKEEKSKHSEQDELMADISKRIQSLEDESKSLKSQVAEAKMTFKIFQMNEERLKIAIKDALNENSQLQESQKQLLQEAEVWKEQVSELNKQKVTFEDSKVHAEQVLNDKESHIKTLTERLLKMKDWAAMLGEDITDDDNLELEMNSESENGAYLDNPPKGALKKLIHAAKLNASLKTLEGERNQIYIQLSEVDKTKEELTEHIKNLQTEQASLQSENTHFENENQKLQQKLKVMTELYQENEMKLHRKLTVEENYRLEKEEKLSKVDEKISHATEELETYRKRAKDLEEELERTIHSYQGQIISHEKKAHDNWLAARNAERNLNDLRKENAHNRQKLTETELKFELLEKDPYALDVPNTAFGREHSPYGPSPLGWPSSETRAFLSPPTLLEGPLRLSPLLPGGGGRGSRGPGNPLDHQITNERGESSCDRLTDPHRAPSDTGSLSPPWDQDRRMMFPPPGQSYPDSALPPQRQDRFCSNSGRLSGPAELRSFNMPSLDKMDGSMPSEMESSRNDTKDDLGNLNVPDSSLPAENEATGPGFVPPPLAPIRGPLFPVDARGPFLRRGPPFPPPPPGAMFGASRDYFPPGDFPGPPPAPFAMRNVYPPRGFPPYLPPRPGFFPPPPHSEGRSEFPSGLIPPSNEPATEHPEPQQET

SEQ ID NO: 416 - protein, 792 aa, synthetic construct
MELKSPEEEVVAALPEGMRPDSNLYGFPWELVICAAVVGFFAVLFFLWRSFRSVRSRLYVGREKKLALMLSGLIEEKSKLLEKFSLVQKEYEGYEVESSLKDASFEKEATEAQSLEATCEKLNRSNSELEDEILCLEKELKEEKSKHSEQDELMADISKRIQSLEDESKSLKSQVAEAKMTFKIFQMNEERLKIAIKDALNENSQLQESQKQLLQEAEVWKEQVSELNKQKVTFEDSKVHAEQVLNDKESHIKTLTERLLKMKDWAAMLGEDITDDDNLELEMNSESENGAYLDNPPKGALKKLIHAAKLNASLKTLEGERNQIYIQLSEVDKTKEELTEHIKNLQTEQASLQSENTHFENENQKLQQKLKVMTELYQENEMKLHRKLTVEENYRLEKEEKLSKVDEKISHATEELETYRKRAKDLEEELERTIHSYQGQIISHEKKAHDNWLAARNAERNLNDLRKENAHNRQKLTETELKFELLEKDPYALDVPNTAFGREHSPYGPSPLGWPSSETRAFLSPPTLLEGPLRLSPLLPGGGGRGSRGPGNPLDHQITNERGESSCDRLTDPHRAPSDTGSLSPPWDQDRRMMFPPPGQSYPDSALPPQRQDRFCSNSGRLSGPAELRSFNMPSLDKMDGSMPSEMESSRNDTKDDLGNLNVPDSSLPAENEATGPGFVPPPLAPIRGPLFPVDARGPFLRRGPPFPPPPPGAMFGASRDYFPPGDFPGPPPAPFAMRNVYPPRGFPPYLPPRPGFFPPPPHSEGRSEFPSGLIPPSNEPATEHPEPQQET

SEQ ID NO: 417 - protein, 330 aa, synthetic construct
ASTKGPSVFPLAPSSKSTSGGTAALGCLVKDYFPEPVTVSWNSGALTSGVHTFPAVLQSSGLYSLSSVVTVPSSSLGTQTYICNVNHKPSNTKVDKRVEPKSCDKTHTCPPCPAPELLGGPSVFLFPPKPKDTLMISRTPEVTCVVVDVSHEDPEVKFNWYVDGVEVHNAKTKPREEQYNSTYRVVSVLTVLHQDWLNGKEYKCKVSNKALPAPIEKTISKAKGQPREPQVYTLPPSREEMTKNQVSLTCLVKGFYPSDIAVEWESNGQPENNYKTTPPVLDSDGSFFLYSKLTVDKSRWQQGNVFSCSVMHEALHNHYTQKSLSLSPGK

SEQ ID NO: 418 - protein, 107 aa, synthetic construct [sequence omitted]